European Patent Specification EP 3 526 605 B1, published November 5, 2025. Title: METHOD FOR THE DETECTION OF APOLIPOPROTEIN E4. Applicant: sphingotec GmbH. The sequence listing filed with the application follows.

SEQUENCE LISTING (15 sequences)

SEQ ID NO: 1 - protein, 299 aa, Homo sapiens
KVEQAVETEPEPELRQQTEWQSGQRWELALGRFWDYLRWVQTLSEQVQEELLSSQVTQELRALMDETMKELKAYKSELEEQLTPVAEETRARLSKELQAAQARLGADMEDVRGRLVQYRGEVQAMLGQSTEELRVRLASHLRKLRKRLLRDADDLQKRLAVYQAGAREGAERGLSAIRERLGPLVEQGRVRAATVGSLAGQPLQERAQAWGERLRARMEEMGSRTRDRLDEVKEQVAEVRAKLEEQAQQIRLQAEAFQARLKSWFEPLVEDMQRQWAGLVEKVQAAVGTSAAPVPSDNH

SEQ ID NO: 2 - protein, 317 aa, Homo sapiens [sequence omitted]

SEQ ID NO: 3 - protein, 165 aa, Homo sapiens
KVEQAVETEPEPELRQQTEWQSGQRWELALGRFWDYLRWVQTLSEQVQEELLSSQVTQELRALMDETMKELKAYKSELEEQLTPVAEETRARLSKELQAAQARLGADMEDVRGRLVQYRGEVQAMLGQSTEELRVRLASHLRKLRKRLLRDADDLQKRLAVYQAG

SEQ ID NO: 4 - protein, 185 aa, Homo sapiens
KVEQAVETEPEPELRQQTEWQSGQRWELALGRFWDYLRWVQTLSEQVQEELLSSQVTQELRALMDETMKELKAYKSELEEQLTPVAEETRARLSKELQAAQARLGADMEDVRGRLVQYRGEVQAMLGQSTEELRVRLASHLRKLRKRLLRDADDLQKRLAVYQAGAREGAERGLSAIRERLGPLV

SEQ ID NO: 5 - protein, 191 aa, Homo sapiens
KVEQAVETEPEPELRQQTEWQSGQRWELALGRFWDYLRWVQTLSEQVQEELLSSQVTQELRALMDETMKELKAYKSELEEQLTPVAEETRARLSKELQAAQARLGADMEDVRGRLVQYRGEVQAMLGQSTEELRVRLASHLRKLRKRLLRDADDLQKRLAVYQAGAREGAERGLSAIRERLGPLVEQGRVR

SEQ ID NO: 6 - protein, 202 aa, Homo sapiens
KVEQAVETEPEPELRQQTEWQSGQRWELALGRFWDYLRWVQTLSEQVQEELLSSQVTQELRALMDETMKELKAYKSELEEQLTPVAEETRARLSKELQAAQARLGADMEDVRGRLVQYRGEVQAMLGQSTEELRVRLASHLRKLRKRLLRDADDLQKRLAVYQAGAREGAERGLSAIRERLGPLVEQGRVRAATVGSLAGQP

SEQ ID NO: 7 - protein, 229 aa, Homo sapiens
KVEQAVETEPEPELRQQTEWQSGQRWELALGRFWDYLRWVQTLSEQVQEELLSSQVTQELRALMDETMKELKAYKSELEEQLTPVAEETRARLSKELQAAQARLGADMEDVRGRLVQYRGEVQAMLGQSTEELRVRLASHLRKLRKRLLRDADDLQKRLAVYQAGAREGAERGLSAIRERLGPLVEQGRVRAATVGSLAGQPLQERAQAWGERLRARMEEMGSRTRDRL

SEQ ID NO: 8 - protein, 231 aa, Homo sapiens
KVEQAVETEPEPELRQQTEWQSGQRWELALGRFWDYLRWVQTLSEQVQEELLSSQVTQELRALMDETMKELKAYKSELEEQLTPVAEETRARLSKELQAAQARLGADMEDVRGRLVQYRGEVQAMLGQSTEELRVRLASHLRKLRKRLLRDADDLQKRLAVYQAGAREGAERGLSAIRERLGPLVEQGRVRAATVGSLAGQPLQERAQAWGERLRARMEEMGSRTRDRLDE

SEQ ID NO: 9 - protein, 251 aa, Homo sapiens
KVEQAVETEPEPELRQQTEWQSGQRWELALGRFWDYLRWVQTLSEQVQEELLSSQVTQELRALMDETMKELKAYKSELEEQLTPVAEETRARLSKELQAAQARLGADMEDVRGRLVQYRGEVQAMLGQSTEELRVRLASHLRKLRKRLLRDADDLQKRLAVYQAGAREGAERGLSAIRERLGPLVEQGRVRAATVGSLAGQPLQERAQAWGERLRARMEEMGSRTRDRLDEVKEQVAEVRAKLEEQAQQIR

SEQ ID NO: 10 - protein, 259 aa, Homo sapiens
KVEQAVETEPEPELRQQTEWQSGQRWELALGRFWDYLRWVQTLSEQVQEELLSSQVTQELRALMDETMKELKAYKSELEEQLTPVAEETRARLSKELQAAQARLGADMEDVRGRLVQYRGEVQAMLGQSTEELRVRLASHLRKLRKRLLRDADDLQKRLAVYQAGAREGAERGLSAIRERLGPLVEQGRVRAATVGSLAGQPLQERAQAWGERLRARMEEMGSRTRDRLDEVKEQVAEVRAKLEEQAQQIRLQAEAFQA

SEQ ID NO: 11 - protein, 260 aa, Homo sapiens
KVEQAVETEPEPELRQQTEWQSGQRWELALGRFWDYLRWVQTLSEQVQEELLSSQVTQELRALMDETMKELKAYKSELEEQLTPVAEETRARLSKELQAAQARLGADMEDVRGRLVQYRGEVQAMLGQSTEELRVRLASHLRKLRKRLLRDADDLQKRLAVYQAGAREGAERGLSAIRERLGPLVEQGRVRAATVGSLAGQPLQERAQAWGERLRARMEEMGSRTRDRLDEVKEQVAEVRAKLEEQAQQIRLQAEAFQAR

SEQ ID NO: 12 - protein, 266 aa, Homo sapiens
KVEQAVETEPEPELRQQTEWQSGQRWELALGRFWDYLRWVQTLSEQVQEELLSSQVTQELRALMDETMKELKAYKSELEEQLTPVAEETRARLSKELQAAQARLGADMEDVRGRLVQYRGEVQAMLGQSTEELRVRLASHLRKLRKRLLRDADDLQKRLAVYQAGAREGAERGLSAIRERLGPLVEQGRVRAATVGSLAGQPLQERAQAWGERLRARMEEMGSRTRDRLDEVKEQVAEVRAKLEEQAQQIRLQAEAFQARLKSWFE

SEQ ID NO: 13 - protein, 271 aa, Homo sapiens
KVEQAVETEPEPELRQQTEWQSGQRWELALGRFWDYLRWVQTLSEQVQEELLSSQVTQELRALMDETMKELKAYKSELEEQLTPVAEETRARLSKELQAAQARLGADMEDVRGRLVQYRGEVQAMLGQSTEELRVRLASHLRKLRKRLLRDADDLQKRLAVYQAGAREGAERGLSAIRERLGPLVEQGRVRAATVGSLAGQPLQERAQAWGERLRARMEEMGSRTRDRLDEVKEQVAEVRAKLEEQAQQIRLQAEAFQARLKSWFEPLVED

SEQ ID NO: 14 - protein, 272 aa, Homo sapiens
KVEQAVETEPEPELRQQTEWQSGQRWELALGRFWDYLRWVQTLSEQVQEELLSSQVTQELRALMDETMKELKAYKSELEEQLTPVAEETRARLSKELQAAQARLGADMEDVRGRLVQYRGEVQAMLGQSTEELRVRLASHLRKLRKRLLRDADDLQKRLAVYQAGAREGAERGLSAIRERLGPLVEQGRVRAATVGSLAGQPLQERAQAWGERLRARMEEMGSRTRDRLDEVKEQVAEVRAKLEEQAQQIRLQAEAFQARLKSWFEPLVEDM

SEQ ID NO: 15 - protein, 228 aa, Homo sapiens
KAYKSELEEQLTPVAEETRARLSKELQAAQARLGADMEDVRGRLVQYRGEVQAMLGQSTEELRVRLASHLRKLRKRLLRDADDLQKRLAVYQAGAREGAERGLSAIRERLGPLVEQGRVRAATVGSLAGQPLQERAQAWGERLRARMEEMGSRTRDRLDEVKEQVAEVRAKLEEQAQQIRLQAEAFQARLKSWFEPLVEDMQRQWAGLVEKVQAAVGTSAAPVPSDNH